European Patent Specification EP 3 279 316 B1, published September 20, 2023. Title: CORTICOSPINAL UPPER MOTOR NEURONS, METHODS AND COMPOSITIONS FOR DIFFERENTIATING NEURAL STEM CELLS BY MODULATING CB1 CANNABINOID RECEPTOR SIGNALING AND USES THEREOF. Applicant: Centro de Investigación Biomédica en Red de Enfermedades Neurodegenerativas- CIBERNED Universidad Complutense de Madrid. The sequence listing filed with the application follows.

SEQUENCE LISTING (2 sequences)

SEQ ID NO: 1 - DNA, 19 bp, Artificial Sequence
  Clim1 forward primer
accctcattccccgttatt

SEQ ID NO: 2 - DNA, 19 bp, Artificial Sequence
  Clim1 reverse primer
tggctctcctaccaccatc